European Patent Specification EP 3 908 322 B1, published August 26, 2026. Title: CELL PENETRATING PEPTIDES. Applicant: University of Tartu. The sequence listing filed with the application follows.

SEQUENCE LISTING (21 sequences)

SEQ ID NO: 1 - protein, 21 aa, Artificial Sequence
  Cell penetrating amino acid sequence; NF55
  MISC_FEATURE (7)..(7): Xaa = Orn; the peptide continues from the side chain amino group and not from the alpha-amino group
AGYLLGXINLKALAALAKAIL

SEQ ID NO: 2 - protein, 21 aa, Artificial Sequence
  Cell penetrating amino acid sequence; NF71, N712, NF713, NF717
  MISC_FEATURE (7)..(7): Xaa = Orn; the peptide continues from the side chain amino group and not from the alpha-amino group
HHYHHGXILLKALKALAKAIL

SEQ ID NO: 3 - protein, 23 aa, Artificial Sequence
  Cell penetrating amino acid sequence; NF70, NF703, NF702, NF701, NF700, NF711
  MISC_FEATURE (9)..(9): Xaa = Orn; the peptide continues from the side chain amino group and not from the alpha-amino group
HHHHYHHGXILLKALKALAKAIL

SEQ ID NO: 4 - protein, 22 aa, Artificial Sequence
  Cell penetrating amino acid sequence; NF704, NF705, NF706
  MISC_FEATURE (8)..(8): Xaa = Orn; the peptide continues from the side chain amino group and not from the alpha-amino group
HHHHHHGXILLKALKALAKAIL

SEQ ID NO: 5 - protein, 25 aa, Artificial Sequence
  Cell penetrating amino acid sequence; NF72, NF721, NF722
  MISC_FEATURE (11)..(11): Xaa = Orn; the peptide continues from the side chain amino group and not from the alpha-amino group
HHHHHHYHHGXILLKALKALAKAIL

SEQ ID NO: 6 - protein, 20 aa, Artificial Sequence
  General formula of the cell penentrating amino acid sequence of the invention
  MISC_FEATURE (6)..(6): Xaa = Orn; the peptide continues from the side chain amino group and not from the alpha-amino group
HYHHGXILLKALKALAKAIL

SEQ ID NO: 7 - DNA, 21 bp, Artificial Sequence
  siRNA sense strand against luc2
ggacgaggacgagcacuuctt

SEQ ID NO: 8 - RNA, 21 nt, Artificial Sequence
  siRNA antisense strand against luc2
gaagugcucguccucguccuu

SEQ ID NO: 9 - RNA, 21 nt, Artificial Sequence
  siRNA sense strand against GFP
ggcuacguccaggagcgcacc

SEQ ID NO: 10 - RNA, 21 nt, Artificial Sequence
  siRNA antisense strand against GFP
ugcgcuccuggacguagccuu

SEQ ID NO: 11 - DNA, 21 bp, Artificial Sequence
  Mus blood coagulation factor VII forward PCR primer
acaagtcttacgtctgcttct

SEQ ID NO: 12 - DNA, 21 bp, Artificial Sequence
  Mus blood coagulation factor VII reverse PCR primer
cacagatcagctgctcattct

SEQ ID NO: 13 - DNA, 20 bp, Artificial Sequence
  Mus Actin beta forward PCR primer
ccacacccgccaccagttcg

SEQ ID NO: 14 - DNA, 20 bp, Artificial Sequence
  Mus Actin beta reverse PCR primer
tacagcccggggagcatcgt

SEQ ID NO: 15 - protein, 25 aa, Artificial Sequence
  Cell penetrating amino acid sequence; NF707, NF708, NF709
  MISC_FEATURE (11)..(11): Xaa = Orn; the peptide continues from the side chain amino group and not from the alpha amino group
HHHHHHYLLGXILLKALKALAKAIL

SEQ ID NO: 16 - protein, 21 aa, Artificial Sequence
  Cell penetrating amino acid sequence of Figure 12, NF714
  MISC_FEATURE (7)..(7): Xaa = Orn; the peptide continues from the side chain amino group and not from the alpha-amino group
HHYHHGXINLKALKALAKAIL

SEQ ID NO: 17 - protein, 21 aa, Artificial Sequence
  Cell penetrating amino acid sequence of Figure 12, NF73
  MISC_FEATURE (7)..(7): Xaa = Orn; the peptide continues from the side chain amino group and not from the alpha-amino group
AGYLLGXIHLKAHKAHAKAHL

SEQ ID NO: 18 - protein, 21 aa, Artificial Sequence
  Cell penetrating amino acid sequence of Figure 12, NF74
  MISC_FEATURE (7)..(7): Xaa = Orn; the peptide continues from the side chain amino group and not from the alpha-amino group
AGYLLGXILHKAHHKLHKAIL

SEQ ID NO: 19 - protein, 20 aa, Artificial Sequence
  Cell penetrating amino acid sequence of the invention; NF725, NF726, NF727
  MISC_FEATURE (6)..(6): Xaa = Orn; the peptide continues from the side chain amino group and not from the alpha-amino group
HYHHGXILLKALKALAKAIL

SEQ ID NO: 20 - protein, 22 aa, Artificial Sequence
  Cell penetrating amino acid sequence of the invention; NF715, NF716, NF718
  MISC_FEATURE (8)..(8): Xaa = Orn; the peptide continues from the side chain amino group and not from the alpha-amino group
HHHYHHGXILLKALKALAKAIL

SEQ ID NO: 21 - protein, 24 aa, Artificial Sequence
  Cell penetrating amino acid sequence of the invention; NF719, NF723, NF724
  MISC_FEATURE (10)..(10): Xaa = Orn; the peptide continues from the side chain amino group and not from the alpha-amino group
HHHHHYHHGXILLKALKALAKAIL